European Patent Specification EP 4 034 885 B1, published August 21, 2024. Title: METHOD FOR DETERMINING POTENCY OF THERAPEUTICAL ANTI-CLEVER-1 ANTIBODY,. Applicant: Faron Pharmaceuticals Oy. The sequence listing filed with the application follows.

SEQUENCE LISTING (15 sequences)

SEQ ID NO: 1 - protein, 15 aa, Homo sapiens
PFTVLVPSVSSFSSR

SEQ ID NO: 2 - protein, 12 aa, Homo sapiens
QEITVTFNQFTK

SEQ ID NO: 3 - protein, 10 aa, Homo sapiens
ATQTGRVFLQ

SEQ ID NO: 4 - protein, 12 aa, Homo sapiens
DSLRDGRLIYLF

SEQ ID NO: 5 - protein, 13 aa, Homo sapiens
SKGRILTMANQVL

SEQ ID NO: 6 - protein, 15 aa, Homo sapiens
LCVYQKPGQAFCTCR

SEQ ID NO: 7 - protein, 1051 aa, Homo sapiens
LCCACLLELIPYAPTLSWTACPPAMAGPRGLLPLCLLAFCLAGFSFVRGQVLFKGCDVKTTFVTHVPCTSCAAIKKQTCPSGWLRELPDQITQDCRYEVQLGGSMVSMSGCRRKCRKQVVQKACCPGYWGSRCHECPGGAETPCNGHGTCLDGMDRNGTCVCQENFRGSACQECQDPNRFGPDCQSVCSCVHGVCNHGPRGDGSCLCFAGYTGPHCDQELPVCQELRCPQNTQCSAEAPSCRCLPGYTQQGSECRAPNPCWPSPCSLLAQCSVSPKGQAQCHCPENYHGDGMVCLPKDPCTDNLGGCPSNSTLCVYQKPGQAFCTCRPGLVSINSNASAGCFAFCSPFSCDRSATCQVTADGKTSCVCRESEVGDGRACYGHLLHEVQKATQTGRVFLQLRVAVAMMDQGCREILTTAGPFTVLVPSVSSFSSRTMNASLAQQLCRQHIIAGQHILEDTRTQQTRRWWTLAGQEITVTFNQFTKYSYKYKDQPQQTFNIYKANNIAANGVFHVVTGLRWQAPSGTPGDPKRTIGQILASTEAFSRFETILENCGLPSILDGPGPFTVFAPSNEAVDSLRDGRLIYLFTAGLSKLQELVRYHIYNHGQLTVEKLISKGRILTMANQVLAVNISEEGRILLGPEGVPLQRVDVMAANGVIHMLDGILLPPTILPILPKHCSEEQHKIVAGSCVDCQALNTSTCPPNSVKLDIFPKECVYIHDPTGLNVLKKGCASYCNQTIMEQGCCKGFFGPDCTQCPGGFSNPCYGKGNCSDGIQGNGACLCFPDYKGIACHICSNPNKHGEQCQEDCGCVHGLCDNRPGSGGVCQQGTCAPGFSGRFCNESMGDCGPTGLAQHCHLHARCVSQEGVARCRCLDGFEGDGFSCTPSNPCSHPDRGGCSENAECVPGSLGTHHCTCHKGWSGDGRVCVAIDECELDMRGGCHTDALCSYVGPGQSRCTCKLGFAGDGYQCSPIDPCRAGNGGCHGLATCRAVGGGQRVCTCPPGFGGDGFSCYGDIFRELEANAHFSIFYQWLKSAGITLPADRRVTALVPS

SEQ ID NO: 8 - protein, 449 aa, Homo sapiens
QVTLKESGPTLVKPTQTLTLTCSFSGFSLSTSGMGIGWIRQPPGKALEWLAHIWWDDDKRYNPALKSRLTISKDTSKNQVVLTMTNMDPVDTATYYCARHYGYDPYYAMDYWGQGTLVTVSSASTKGPSVFPLAPCSRSTSESTAALGCLVKDYFPEPVTVSWNSGALTSGVHTFPAVLQSSGLYSLSSVVTVPSSSLGTKTYTCNVDHKPSNTKVDKRVESKYGPPCPPCPAPEFEGGPSVFLFPPKPKDTLMISRTPEVTCVVVDVSQEDPEVQFNWYVDGVEVHNAKTKPREEQFNSTYRVVSVLTVLHQDWLNGKEYKCKVSNKGLPSSIEKTISKAKGQPREPQVYTLPPSQEEMTKNQVSLTCLVKGFYPSDIAVEWESNGQPENNYKTTPPVLDSDGSFFLYSRLTVDKSRWQEGNVFSCSVMHEALHNHYTQKSLSLSLGK

SEQ ID NO: 9 - protein, 215 aa, Homo sapiens
EIVLTQSPGTLSLSPGERATLSCTASSSVSSSYLHWYQQKPGKAPKLLIYRTSNLASGVPSRFSGSGSGTDYTLTISSLQPEDFATYYCHQYHRSPPTFGQGTKLEIKRTVAAPSVFIFPPSDEQLKSGTASVVCLLNNFYPREAKVQWKVDNALQSGNSQESVTEQDKSDSTYSLSSTLTLSKADYEKHKVYACEVTHQGLSSPVTKSFNRGEC

SEQ ID NO: 10 - protein, 7 aa, Homo sapiens
TSGMGIG

SEQ ID NO: 11 - protein, 16 aa, Homo sapiens
HIWWDDDKRYNPALKS

SEQ ID NO: 12 - protein, 12 aa, Homo sapiens
HYGYDPYYAMDY

SEQ ID NO: 13 - protein, 12 aa, Homo sapiens
TASSSVSSSYLH

SEQ ID NO: 14 - protein, 7 aa, Homo sapiens
RTSNLAS

SEQ ID NO: 15 - protein, 9 aa, Homo sapiens
HQYHRSPPT